European Patent Application EP 4 282 954 A1, published November 29, 2023. Title: CELL STRAIN FOR PRODUCING BIOSIMILAR DRUG OF USTEKINUMAB AND PRODUCTION METHOD THEREFOR. Applicant: Qyuns Therapeutics Co., Ltd. The sequence listing filed with the application follows.

SEQUENCE LISTING (4 sequences)

SEQ ID NO: 1 - protein, 449 aa, Artificial sequence
  Artificial
EVQLVQSGAEVKKPGESLKISCKGSGYSFTTYWLGWVRQMPGKGLDWIGIMSPVDSDIRYSPSFQGQVTMSVDKSITTAYLQWNSLKASDTAMYYCARRRPGQGYFDFWGQGTLVTVSSSSTKGPSVFPLAPSSKSTSGGTAALGCLVKDYFPEPVTVSWNSGALTSGVHTFPAVLQSSGLYSLSSVVTVPSSSLGTQTYICNVNHKPSNTKVDKRVEPKSCDKTHTCPPCPAPELLGGPSVFLFPPKPKDTLMISRTPEVTCVVVDVSHEDPEVKFNWYVDGVEVHNAKTKPREEQYNSTYRVVSVLTVLHQDWLNGKEYKCKVSNKALPAPIEKTISKAKGQPREPQVYTLPPSRDELTKNQVSLTCLVKGFYPSDIAVEWESNGQPENNYKTTPPVLDSDGSFFLYSKLTVDKSRWQQGNVFSCSVMHEALHNHYTQKSLSLSPGK

SEQ ID NO: 2 - DNA, 1347 bp, Artificial sequence
  Artificial
gaagtccagctggtgcagtcaggggccgaggtgaagaaaccaggtgaaagtctgaagatcagctgtaaaggctctggatacagtttcaccacatattggctgggatgggtgcggcagatgcccgggaagggtctggattggatcggtattatgtcccccgtggacagcgacatcagatacagtccttcatttcagggccaggtcactatgtctgtggacaagagtattactaccgcttatctgcagtggaactcactgaaagcctccgataccgctatgtactattgcgcaaggcggagacccggccagggatacttcgacttttgggggcagggcaccctggtcacagtgtccagctctagtactaaggggccttccgtgtttccactggctccctcatccaaatccactagcggaggaaccgcagctctgggatgtctggtgaaggactatttcccagagcccgtcacagtgtcatggaactccggcgcactgaccagcggagtccatacatttcctgccgtgctgcagagctctgggctgtactctctgagttcagtggtcacagtgccatccagctctctgggtactcagacctatatctgcaacgtgaatcacaagccttctaatactaaggtcgataagagggtggaaccaaagagttgtgataaaacacatacttgccccccttgtcctgcaccagagctgctggggggtccaagcgtgttcctgtttccacccaagcccaaagataccctgatgatttcccgaacaccagaagtcacttgcgtggtcgtggacgtgagccacgaggaccccgaagtcaagttcaactggtacgtggacggcgtcgaggtgcataatgctaagaccaaacctcgcgaggaacagtacaatagcacatatcgagtcgtgtctgtcctgactgtgctgcaccaggattggctgaacggaaaggagtataagtgcaaagtgtctaataaggctctgcccgcacctatcgagaaaaccatttccaaggccaaaggccagcctcgtgaaccacaggtgtacacactgcctccatcaagggatgagctgactaagaaccaagtcagcctgacctgtctggtgaaaggcttctatccctctgacatcgctgtggagtgggaaagtaatggacagcctgaaaacaattacaagacaactccccctgtgctggacagcgatggctctttctttctgtattccaagctgaccgtggacaaaagccggtggcagcagggaaacgtcttttcttgtagtgtgatgcatgaggccctgcacaatcattacacacagaagtcactgtccctgagcccaggaaaa

SEQ ID NO: 3 - protein, 214 aa, Artificial sequence
  Artificial
DIQMTQSPSSLSASVGDRVTITCRASQGISSWLAWYQQKPEKAPKSLIYAASSLQSGVPSRFSGSGSGTDFTLTISSLQPEDFATYYCQQYNIYPYTFGQGTKLEIKRTVAAPSVFIFPPSDEQLKSGTASVVCLLNNFYPREAKVQWKVDNALQSGNSQESVTEQDSKDSTYSLSSTLTLSKADYEKHKVYACEVTHQGLSSPVTKSFNRGEC

SEQ ID NO: 4 - DNA, 642 bp, Artificial sequence
  Artificial
gacatccagatgacccagagtccatccagcctgtctgctagtgtgggagatagggtcactatcacctgtcgggcctcccaggggatttctagttggctggcttggtatcagcagaagccagagaaagcacccaagtccctgatttatgccgcttcatccctgcagagtggagtgccctcacgattctcaggctccggaagcgggactgactttacactgactatcagctctctgcagcctgaagatttcgctacctactattgccagcagtacaacatttacccatatacttttggtcagggcaccaaactggagatcaagagaacagtggcagcccccagcgtcttcatttttcccccttctgacgaacagctgaaatccggcaccgcaagcgtggtctgtctgctgaacaatttctaccctcgcgaggccaaagtgcagtggaaggtcgataacgctctgcagtctggcaatagtcaggagtcagtgacagaacaggactccaaagatagcacttattctctgagttcaaccctgacactgagcaaggcagactacgagaagcacaaagtgtatgcctgcgaagtcacccatcagggtctgtccagccccgtgacaaagtcttttaataggggcgaatgt